European Patent Application EP 4 524 160 A2, published March 19, 2025. Title: COMPOSITIONS AND METHODS FOR THE MODULATION OF BETA CHAIN-MEDIATED IMMUNITY. Applicant: Janssen Biotech, Inc. The sequence listing filed with the application follows.

SEQUENCE LISTING (440 sequences)

SEQ ID NO: 1 - protein, 5 aa, synthetic construct
  REGION 1..5: note = synthetic construct
SYGVH

SEQ ID NO: 2 - protein, 16 aa, synthetic construct
  REGION 1..16: note = synthetic construct
IIWSAGGTDYNAAFIS

SEQ ID NO: 3 - protein, 11 aa, synthetic construct
  REGION 1..11: note = synthetic construct
GSFYDYGRLDY

SEQ ID NO: 4 - protein, 11 aa, synthetic construct
  REGION 1..11: note = synthetic construct
KASQDVSTAVA

SEQ ID NO: 5 - protein, 7 aa, synthetic construct
  REGION 1..7: note = synthetic construct
SSSYRYT

SEQ ID NO: 6 - protein, 9 aa, synthetic construct
  REGION 1..9: note = synthetic construct
QQHYGTPYT

SEQ ID NO: 7 - protein, 7 aa, synthetic construct
  REGION 1..7: note = synthetic construct
GFSLTSY

SEQ ID NO: 8 - protein, 5 aa, synthetic construct
  REGION 1..5: note = synthetic construct
WSAGG

SEQ ID NO: 9 - protein, 11 aa, synthetic construct
  REGION 1..11: note = synthetic construct
GSFYDYGRLDY

SEQ ID NO: 10 - protein, 11 aa, synthetic construct
  REGION 1..11: note = synthetic construct
KASQDVSTAVA

SEQ ID NO: 11 - protein, 7 aa, synthetic construct
  REGION 1..7: note = synthetic construct
SSSYRYT

SEQ ID NO: 12 - protein, 9 aa, synthetic construct
  REGION 1..9: note = synthetic construct
QQHYGTPYT

SEQ ID NO: 13 - protein, 10 aa, synthetic construct
  REGION 1..10: note = synthetic construct
GFSLTSYGVH

SEQ ID NO: 14 - protein, 9 aa, synthetic construct
  REGION 1..9: note = synthetic construct
IIWSAGGTD

SEQ ID NO: 15 - protein, 11 aa, synthetic construct
  REGION 1..11: note = synthetic construct
GSFYDYGRLDY

SEQ ID NO: 16 - protein, 11 aa, synthetic construct
  REGION 1..11: note = synthetic construct
KASQDVSTAVA

SEQ ID NO: 17 - protein, 7 aa, synthetic construct
  REGION 1..7: note = synthetic construct
SSSYRYT

SEQ ID NO: 18 - protein, 9 aa, synthetic construct
  REGION 1..9: note = synthetic construct
QQHYGTPYT

SEQ ID NO: 19 - protein, 6 aa, synthetic construct
  REGION 1..6: note = synthetic construct
TSYGVH

SEQ ID NO: 20 - protein, 12 aa, synthetic construct
  REGION 1..12: note = synthetic construct
WLGIIWSAGGTD

SEQ ID NO: 21 - protein, 12 aa, synthetic construct
  REGION 1..12: note = synthetic construct
ARGSFYDYGRLD

SEQ ID NO: 22 - protein, 7 aa, synthetic construct
  REGION 1..7: note = synthetic construct
STAVAWY

SEQ ID NO: 23 - protein, 10 aa, synthetic construct
  REGION 1..10: note = synthetic construct
LLIYSSSYRY

SEQ ID NO: 24 - protein, 8 aa, synthetic construct
  REGION 1..8: note = synthetic construct
QQHYGTPY

SEQ ID NO: 25 - protein, 8 aa, synthetic construct
  REGION 1..8: note = synthetic construct
GFSLTSYG

SEQ ID NO: 26 - protein, 7 aa, synthetic construct
  REGION 1..7: note = synthetic construct
IWSAGGT

SEQ ID NO: 27 - protein, 13 aa, synthetic construct
  REGION 1..13: note = synthetic construct
ARGSFYDYGRLDY

SEQ ID NO: 28 - protein, 6 aa, synthetic construct
  REGION 1..6: note = synthetic construct
QDVSTA

SEQ ID NO: 29 - skipped

SEQ ID NO: 30 - protein, 9 aa, synthetic construct
  REGION 1..9: note = synthetic construct
QQHYGTPYT

SEQ ID NO: 31 - protein, 119 aa, synthetic construct
  REGION 1..119: note = synthetic construct
EVQLQESGPGLVQPSQSLSITCTVSGFSLTSYGVHWVRQSPGKGLEWLGIIWSAGGTDYNAAFISRLSISKDNSKSQIFFKLNSLHADDTAIYFCARGSFYDYGRLDYWGQGTTLTVSS

SEQ ID NO: 32 - protein, 107 aa, synthetic construct
  REGION 1..107: note = synthetic construct
DIVMTQSHRFMSTSVGDRVSITCKASQDVSTAVAWYQQKPGQSPKLLIYSSSYRYTGVPDRFTGSGSGTDFTFTISSVQAEDLAVYYCQQHYGTPYTFGGGTKLEIQ

SEQ ID NO: 33-34 - skipped (2 entries)

SEQ ID NO: 35 - protein, 5 aa, synthetic construct
  REGION 1..5: note = synthetic construct
HYWID

SEQ ID NO: 36 - protein, 17 aa, synthetic construct
  REGION 1..17: note = synthetic construct
NIYPGGGYTNYNENFKG

SEQ ID NO: 37 - protein, 13 aa, synthetic construct
  REGION 1..13: note = synthetic construct
KGYYYGSDWYFDV

SEQ ID NO: 38 - protein, 11 aa, synthetic construct
  REGION 1..11: note = synthetic construct
KASQDVSTAVA

SEQ ID NO: 39 - protein, 7 aa, synthetic construct
  REGION 1..7: note = synthetic construct
SASYRYT

SEQ ID NO: 40 - protein, 9 aa, synthetic construct
  REGION 1..9: note = synthetic construct
QQHYTTPYT

SEQ ID NO: 41 - protein, 7 aa, synthetic construct
  REGION 1..7: note = synthetic construct
GYTFTHY

SEQ ID NO: 42 - protein, 6 aa, synthetic construct
  REGION 1..6: note = synthetic construct
YPGGGY

SEQ ID NO: 43 - protein, 13 aa, synthetic construct
  REGION 1..13: note = synthetic construct
KGYYYGSDWYFDV

SEQ ID NO: 44 - protein, 11 aa, synthetic construct
  REGION 1..11: note = synthetic construct
KASQDVSTAVA

SEQ ID NO: 45 - protein, 7 aa, synthetic construct
  REGION 1..7: note = synthetic construct
SASYRYT

SEQ ID NO: 46 - protein, 9 aa, synthetic construct
  REGION 1..9: note = synthetic construct
QQHYTTPYT

SEQ ID NO: 47 - protein, 10 aa, synthetic construct
  REGION 1..10: note = synthetic construct
GYTFTHYWID

SEQ ID NO: 48 - protein, 10 aa, synthetic construct
  REGION 1..10: note = synthetic construct
NIYPGGGYTN

SEQ ID NO: 49 - protein, 13 aa, synthetic construct
  REGION 1..13: note = synthetic construct
KGYYYGSDWYFDV

SEQ ID NO: 50 - protein, 11 aa, synthetic construct
  REGION 1..11: note = synthetic construct
KASQDVSTAVA

SEQ ID NO: 51 - protein, 7 aa, synthetic construct
  REGION 1..7: note = synthetic construct
SASYRYT

SEQ ID NO: 52 - protein, 9 aa, synthetic construct
  REGION 1..9: note = synthetic construct
QQHYTTPYT

SEQ ID NO: 53 - protein, 6 aa, synthetic construct
  REGION 1..6: note = synthetic construct
THYWID

SEQ ID NO: 54 - protein, 13 aa, synthetic construct
  REGION 1..13: note = synthetic construct
WIGNIYPGGGYTN

SEQ ID NO: 55 - protein, 14 aa, synthetic construct
  REGION 1..14: note = synthetic construct
TRKGYYYGSDWYFD

SEQ ID NO: 56 - protein, 7 aa, synthetic construct
  REGION 1..7: note = synthetic construct
STAVAWY

SEQ ID NO: 57 - protein, 10 aa, synthetic construct
  REGION 1..10: note = synthetic construct
LLIYSASYRY

SEQ ID NO: 58 - protein, 8 aa, synthetic construct
  REGION 1..8: note = synthetic construct
QQHYTTPY

SEQ ID NO: 59 - protein, 8 aa, synthetic construct
  REGION 1..8: note = synthetic construct
GYTFTHYW

SEQ ID NO: 60 - protein, 8 aa, synthetic construct
  REGION 1..8: note = synthetic construct
IYPGGGYT

SEQ ID NO: 61 - protein, 15 aa, synthetic construct
  REGION 1..15: note = synthetic construct
TRKGYYYGSDWYFDV

SEQ ID NO: 62 - protein, 6 aa, synthetic construct
  REGION 1..6: note = synthetic construct
QDVSTA

SEQ ID NO: 63 - skipped

SEQ ID NO: 64 - protein, 9 aa, synthetic construct
  REGION 1..9: note = synthetic construct
QQHYTTPYT

SEQ ID NO: 65 - protein, 122 aa, synthetic construct
  REGION 1..122: note = synthetic construct
EVQLQESGAELVRPGTSVKMSCKASGYTFTHYWIDWTKQRPGHGLEWIGNIYPGGGYTNYNENFKGKATLTADKSSSTVFMQFSSLTSDDSAIYYCTRKGYYYGSDWYFDVWGTGTTVTVSS

SEQ ID NO: 66 - protein, 96 aa, synthetic construct
  REGION 1..96: note = synthetic construct
STSVGDRVSITCKASQDVSTAVAWYHQKPGQSPKLLIYSASYRYTGVPDRFTGSGSGTDFTFTISSVQAEDLAVYYCQQHYTTPYTFGGGTKLEMK

SEQ ID NO: 67-68 - skipped (2 entries)

SEQ ID NO: 69 - protein, 5 aa, synthetic construct
  REGION 1..5: note = synthetic construct
TYGMN

SEQ ID NO: 70 - protein, 17 aa, synthetic construct
  REGION 1..17: note = synthetic construct
YLNTYSGVSTYADDFKG

SEQ ID NO: 71 - protein, 9 aa, synthetic construct
  REGION 1..9: note = synthetic construct
WGNYGAMDY

SEQ ID NO: 72 - protein, 16 aa, synthetic construct
  REGION 1..16: note = synthetic construct
RSSQSIVRSNGFTYLE

SEQ ID NO: 73 - protein, 7 aa, synthetic construct
  REGION 1..7: note = synthetic construct
KVSNRFS

SEQ ID NO: 74 - protein, 9 aa, synthetic construct
  REGION 1..9: note = synthetic construct
FQSSHVPRT

SEQ ID NO: 75 - protein, 7 aa, synthetic construct
  REGION 1..7: note = synthetic construct
GYTFTTY

SEQ ID NO: 76 - protein, 6 aa, synthetic construct
  REGION 1..6: note = synthetic construct
NTYSGV

SEQ ID NO: 77 - protein, 9 aa, synthetic construct
  REGION 1..9: note = synthetic construct
WGNYGAMDY

SEQ ID NO: 78 - protein, 16 aa, synthetic construct
  REGION 1..16: note = synthetic construct
RSSQSIVRSNGFTYLE

SEQ ID NO: 79 - protein, 7 aa, synthetic construct
  REGION 1..7: note = synthetic construct
KVSNRFS

SEQ ID NO: 80 - protein, 9 aa, synthetic construct
  REGION 1..9: note = synthetic construct
FQSSHVPRT

SEQ ID NO: 81 - protein, 10 aa, synthetic construct
  REGION 1..10: note = synthetic construct
GYTFTTYGMN

SEQ ID NO: 82 - protein, 10 aa, synthetic construct
  REGION 1..10: note = synthetic construct
YLNTYSGVST

SEQ ID NO: 83 - protein, 9 aa, synthetic construct
  REGION 1..9: note = synthetic construct
WGNYGAMDY

SEQ ID NO: 84 - protein, 16 aa, synthetic construct
  REGION 1..16: note = synthetic construct
RSSQSIVRSNGFTYLE

SEQ ID NO: 85 - protein, 7 aa, synthetic construct
  REGION 1..7: note = synthetic construct
KVSNRFS

SEQ ID NO: 86 - protein, 9 aa, synthetic construct
  REGION 1..9: note = synthetic construct
FQSSHVPRT

SEQ ID NO: 87 - protein, 6 aa, synthetic construct
  REGION 1..6: note = synthetic construct
TTYGMN

SEQ ID NO: 88 - protein, 13 aa, synthetic construct
  REGION 1..13: note = synthetic construct
WMGYLNTYSGVST

SEQ ID NO: 89 - protein, 10 aa, synthetic construct
  REGION 1..10: note = synthetic construct
ARWGNYGAMD

SEQ ID NO: 90 - protein, 12 aa, synthetic construct
  REGION 1..12: note = synthetic construct
VRSNGFTYLEWY

SEQ ID NO: 91 - protein, 10 aa, synthetic construct
  REGION 1..10: note = synthetic construct
LLIYKVSNRF

SEQ ID NO: 92 - protein, 8 aa, synthetic construct
  REGION 1..8: note = synthetic construct
FQSSHVPR

SEQ ID NO: 93 - protein, 8 aa, synthetic construct
  REGION 1..8: note = synthetic construct
GYTFTTYG

SEQ ID NO: 94 - protein, 8 aa, synthetic construct
  REGION 1..8: note = synthetic construct
LNTYSGVS

SEQ ID NO: 95 - protein, 11 aa, synthetic construct
  REGION 1..11: note = synthetic construct
ARWGNYGAMDY

SEQ ID NO: 96 - protein, 11 aa, synthetic construct
  REGION 1..11: note = synthetic construct
QSIVRSNGFTY

SEQ ID NO: 97 - skipped

SEQ ID NO: 98 - protein, 9 aa, synthetic construct
  REGION 1..9: note = synthetic construct
FQSSHVPRT

SEQ ID NO: 99 - protein, 118 aa, synthetic construct
  REGION 1..118: note = synthetic construct
EVQLQESGPDLKKPGETVKISCKASGYTFTTYGMNWVKQAPGKGLKWMGYLNTYSGVSTYADDFKGRFAFSLETSANTAYLQINNLRNDDTATYFCARWGNYGAMDYWGQGTSVTVSS

SEQ ID NO: 100 - protein, 112 aa, synthetic construct
  REGION 1..112: note = synthetic construct
DIKMTQSPLSLPVSLGDQASISCRSSQSIVRSNGFTYLEWYLQKPGQSPELLIYKVSNRFSGVPDRFSGSGSGTDFTLKISRVEAEDLGVYYCFQSSHVPRTFGGGTKLEIK

SEQ ID NO: 101-102 - skipped (2 entries)

SEQ ID NO: 103 - protein, 5 aa, synthetic construct
  REGION 1..5: note = synthetic construct
TYGMN

SEQ ID NO: 104 - protein, 17 aa, synthetic construct
  REGION 1..17: note = synthetic construct
YLNTYSGVSTYADDFKG

SEQ ID NO: 105 - protein, 9 aa, synthetic construct
  REGION 1..9: note = synthetic construct
WGNYGAMDY

SEQ ID NO: 106 - protein, 16 aa, synthetic construct
  REGION 1..16: note = synthetic construct
RSSQSIVRSNGFTYLE

SEQ ID NO: 107 - protein, 7 aa, synthetic construct
  REGION 1..7: note = synthetic construct
KVSNRFS

SEQ ID NO: 108 - protein, 9 aa, synthetic construct
  REGION 1..9: note = synthetic construct
FQSSHVPRT

SEQ ID NO: 109 - protein, 7 aa, synthetic construct
  REGION 1..7: note = synthetic construct
GYTFTTY

SEQ ID NO: 110 - protein, 6 aa, synthetic construct
  REGION 1..6: note = synthetic construct
NTYSGV

SEQ ID NO: 111 - protein, 9 aa, synthetic construct
  REGION 1..9: note = synthetic construct
WGNYGAMDY

SEQ ID NO: 112 - protein, 16 aa, synthetic construct
  REGION 1..16: note = synthetic construct
RSSQSIVRSNGFTYLE

SEQ ID NO: 113 - protein, 7 aa, synthetic construct
  REGION 1..7: note = synthetic construct
KVSNRFS

SEQ ID NO: 114 - protein, 9 aa, synthetic construct
  REGION 1..9: note = synthetic construct
FQSSHVPRT

SEQ ID NO: 115 - protein, 10 aa, synthetic construct
  REGION 1..10: note = synthetic construct
GYTFTTYGMN

SEQ ID NO: 116 - protein, 10 aa, synthetic construct
  REGION 1..10: note = synthetic construct
YLNTYSGVST

SEQ ID NO: 117 - protein, 9 aa, synthetic construct
  REGION 1..9: note = synthetic construct
WGNYGAMDY

SEQ ID NO: 118 - protein, 16 aa, synthetic construct
  REGION 1..16: note = synthetic construct
RSSQSIVRSNGFTYLE

SEQ ID NO: 119 - protein, 7 aa, synthetic construct
  REGION 1..7: note = synthetic construct
KVSNRFS

SEQ ID NO: 120 - protein, 9 aa, synthetic construct
  REGION 1..9: note = synthetic construct
FQSSHVPRT

SEQ ID NO: 121 - protein, 6 aa, synthetic construct
  REGION 1..6: note = synthetic construct
TTYGMN

SEQ ID NO: 122 - protein, 13 aa, synthetic construct
  REGION 1..13: note = synthetic construct
WMGYLNTYSGVST

SEQ ID NO: 123 - protein, 10 aa, synthetic construct
  REGION 1..10: note = synthetic construct
ARWGNYGAMD

SEQ ID NO: 124 - protein, 12 aa, synthetic construct
  REGION 1..12: note = synthetic construct
VRSNGFTYLEWY

SEQ ID NO: 125 - protein, 10 aa, synthetic construct
  REGION 1..10: note = synthetic construct
LLIYKVSNRF

SEQ ID NO: 126 - protein, 8 aa, synthetic construct
  REGION 1..8: note = synthetic construct
FQSSHVPR

SEQ ID NO: 127 - protein, 8 aa, synthetic construct
  REGION 1..8: note = synthetic construct
GYTFTTYG

SEQ ID NO: 128 - protein, 8 aa, synthetic construct
  REGION 1..8: note = synthetic construct
LNTYSGVS

SEQ ID NO: 129 - protein, 11 aa, synthetic construct
  REGION 1..11: note = synthetic construct
ARWGNYGAMDY

SEQ ID NO: 130 - protein, 11 aa, synthetic construct
  REGION 1..11: note = synthetic construct
QSIVRSNGFTY

SEQ ID NO: 131 - skipped

SEQ ID NO: 132 - protein, 9 aa, synthetic construct
  REGION 1..9: note = synthetic construct
FQSSHVPRT

SEQ ID NO: 133 - protein, 118 aa, synthetic construct; identical to SEQ ID NO: 99
  REGION 1..118: note = synthetic construct

SEQ ID NO: 134 - protein, 112 aa, synthetic construct
  REGION 1..112: note = synthetic construct
DIVMTQSPLSLPVSLGDQASISCRSSQSIVRSNGFTYLEWYLQKPGQSPELLIYKVSNRFSGVPDRFSGSGSGTDFTLKISRVEAEDLGVYYCFQSSHVPRTFGGGTKLEIK

SEQ ID NO: 135-136 - skipped (2 entries)

SEQ ID NO: 137 - protein, 6 aa, synthetic construct
  REGION 1..6: note = synthetic construct
SGYYWN

SEQ ID NO: 138 - protein, 16 aa, synthetic construct
  REGION 1..16: note = synthetic construct
YITYDGSNNYNPSLKD

SEQ ID NO: 139 - protein, 7 aa, synthetic construct
  REGION 1..7: note = synthetic construct
GGGYVPV

SEQ ID NO: 140 - protein, 11 aa, synthetic construct
  REGION 1..11: note = synthetic construct
RASQNIGTSIH

SEQ ID NO: 141 - protein, 7 aa, synthetic construct
  REGION 1..7: note = synthetic construct
YASESIS

SEQ ID NO: 142 - protein, 9 aa, synthetic construct
  REGION 1..9: note = synthetic construct
HQSHNWPTT

SEQ ID NO: 143 - protein, 8 aa, synthetic construct
  REGION 1..8: note = synthetic construct
GYSITSGY

SEQ ID NO: 144 - protein, 5 aa, synthetic construct
  REGION 1..5: note = synthetic construct
TYDGS

SEQ ID NO: 145 - protein, 7 aa, synthetic construct
  REGION 1..7: note = synthetic construct
GGGYVPV

SEQ ID NO: 146 - protein, 11 aa, synthetic construct
  REGION 1..11: note = synthetic construct
RASQNIGTSIH

SEQ ID NO: 147 - protein, 7 aa, synthetic construct
  REGION 1..7: note = synthetic construct
YASESIS

SEQ ID NO: 148 - protein, 9 aa, synthetic construct
  REGION 1..9: note = synthetic construct
HQSHNWPTT

SEQ ID NO: 149 - protein, 11 aa, synthetic construct
  REGION 1..11: note = synthetic construct
GYSITSGYYWN

SEQ ID NO: 150 - protein, 9 aa, synthetic construct
  REGION 1..9: note = synthetic construct
YITYDGSNN

SEQ ID NO: 151 - protein, 7 aa, synthetic construct
  REGION 1..7: note = synthetic construct
GGGYVPV

SEQ ID NO: 152 - protein, 11 aa, synthetic construct
  REGION 1..11: note = synthetic construct
RASQNIGTSIH

SEQ ID NO: 153 - protein, 7 aa, synthetic construct
  REGION 1..7: note = synthetic construct
YASESIS

SEQ ID NO: 154 - protein, 9 aa, synthetic construct
  REGION 1..9: note = synthetic construct
HQSHNWPTT

SEQ ID NO: 155 - protein, 7 aa, synthetic construct
  REGION 1..7: note = synthetic construct
TSGYYWN

SEQ ID NO: 156 - protein, 12 aa, synthetic construct
  REGION 1..12: note = synthetic construct
WMGYITYDGSNN

SEQ ID NO: 157 - protein, 8 aa, synthetic construct
  REGION 1..8: note = synthetic construct
ARGGGYVP

SEQ ID NO: 158 - protein, 7 aa, synthetic construct
  REGION 1..7: note = synthetic construct
GTSIHWY

SEQ ID NO: 159 - protein, 10 aa, synthetic construct
  REGION 1..10: note = synthetic construct
LLIKYASESI

SEQ ID NO: 160 - protein, 8 aa, synthetic construct
  REGION 1..8: note = synthetic construct
HQSHNWPT

SEQ ID NO: 161 - protein, 9 aa, synthetic construct
  REGION 1..9: note = synthetic construct
GYSITSGYY

SEQ ID NO: 162 - protein, 7 aa, synthetic construct
  REGION 1..7: note = synthetic construct
ITYDGSN

SEQ ID NO: 163 - protein, 9 aa, synthetic construct
  REGION 1..9: note = synthetic construct
ARGGGYVPV

SEQ ID NO: 164 - protein, 6 aa, synthetic construct
  REGION 1..6: note = synthetic construct
QNIGTS

SEQ ID NO: 165 - skipped

SEQ ID NO: 166 - protein, 9 aa, synthetic construct
  REGION 1..9: note = synthetic construct
HQSHNWPTT

SEQ ID NO: 167 - protein, 116 aa, synthetic construct
  REGION 1..116: note = synthetic construct
EVQLQESGPGLVKPSQSLSLTCSVTGYSITSGYYWNWIRQFLGNKLEWMGYITYDGSNNYNPSLKDRISITRDTSKNQFFLNLNSVTTDDTATYYCARGGGYVPVWGTGTTVTVSS

SEQ ID NO: 168 - protein, 106 aa, synthetic construct
  REGION 1..106: note = synthetic construct
IQMTQSPAFLSVSPGERVSFSCRASQNIGTSIHWYQQRTNGSPRLLIKYASESISGIPSRFSGSGSGTDFTLSINSVESEDFADYYCHQSHNWPTTFGAGTKLELK

SEQ ID NO: 169-170 - skipped (2 entries)

SEQ ID NO: 171 - protein, 6 aa, synthetic construct
  REGION 1..6: note = synthetic construct
SGYYWN

SEQ ID NO: 172 - protein, 16 aa, synthetic construct
  REGION 1..16: note = synthetic construct
YITYDGSNNYNPSLKD

SEQ ID NO: 173 - protein, 7 aa, synthetic construct
  REGION 1..7: note = synthetic construct
GGGYVPV

SEQ ID NO: 174 - protein, 11 aa, synthetic construct
  REGION 1..11: note = synthetic construct
RASQNIGTSIH

SEQ ID NO: 175 - protein, 7 aa, synthetic construct
  REGION 1..7: note = synthetic construct
YASESIS

SEQ ID NO: 176 - protein, 9 aa, synthetic construct
  REGION 1..9: note = synthetic construct
HQSHNWPTT

SEQ ID NO: 177 - protein, 8 aa, synthetic construct
  REGION 1..8: note = synthetic construct
GYSITSGY

SEQ ID NO: 178 - protein, 5 aa, synthetic construct
  REGION 1..5: note = synthetic construct
TYDGS

SEQ ID NO: 179 - protein, 7 aa, synthetic construct
  REGION 1..7: note = synthetic construct
GGGYVPV

SEQ ID NO: 180 - protein, 11 aa, synthetic construct
  REGION 1..11: note = synthetic construct
RASQNIGTSIH

SEQ ID NO: 181 - protein, 7 aa, synthetic construct
  REGION 1..7: note = synthetic construct
YASESIS

SEQ ID NO: 182 - protein, 9 aa, synthetic construct
  REGION 1..9: note = synthetic construct
HQSHNWPTT

SEQ ID NO: 183 - protein, 11 aa, synthetic construct
  REGION 1..11: note = synthetic construct
GYSITSGYYWN

SEQ ID NO: 184 - protein, 9 aa, synthetic construct
  REGION 1..9: note = synthetic construct
YITYDGSNN

SEQ ID NO: 185 - protein, 7 aa, synthetic construct
  REGION 1..7: note = synthetic construct
GGGYVPV

SEQ ID NO: 186 - protein, 11 aa, synthetic construct
  REGION 1..11: note = synthetic construct
RASQNIGTSIH

SEQ ID NO: 187 - protein, 7 aa, synthetic construct
  REGION 1..7: note = synthetic construct
YASESIS

SEQ ID NO: 188 - protein, 9 aa, synthetic construct
  REGION 1..9: note = synthetic construct
HQSHNWPTT

SEQ ID NO: 189 - protein, 7 aa, synthetic construct
  REGION 1..7: note = synthetic construct
TSGYYWN

SEQ ID NO: 190 - protein, 12 aa, synthetic construct
  REGION 1..12: note = synthetic construct
WMGYITYDGSNN

SEQ ID NO: 191 - protein, 8 aa, synthetic construct
  REGION 1..8: note = synthetic construct
ARGGGYVP

SEQ ID NO: 192 - protein, 7 aa, synthetic construct
  REGION 1..7: note = synthetic construct
GTSIHWY

SEQ ID NO: 193 - protein, 10 aa, synthetic construct
  REGION 1..10: note = synthetic construct
LLIKYASESI

SEQ ID NO: 194 - protein, 8 aa, synthetic construct
  REGION 1..8: note = synthetic construct
HQSHNWPT

SEQ ID NO: 195 - protein, 9 aa, synthetic construct
  REGION 1..9: note = synthetic construct
GYSITSGYY

SEQ ID NO: 196 - protein, 7 aa, synthetic construct
  REGION 1..7: note = synthetic construct
ITYDGSN

SEQ ID NO: 197 - protein, 9 aa, synthetic construct
  REGION 1..9: note = synthetic construct
ARGGGYVPV

SEQ ID NO: 198 - protein, 6 aa, synthetic construct
  REGION 1..6: note = synthetic construct
QNIGTS

SEQ ID NO: 199 - skipped

SEQ ID NO: 200 - protein, 9 aa, synthetic construct
  REGION 1..9: note = synthetic construct
HQSHNWPTT

SEQ ID NO: 201 - protein, 116 aa, synthetic construct; identical to SEQ ID NO: 167
  REGION 1..116: note = synthetic construct

SEQ ID NO: 202 - protein, 107 aa, synthetic construct
  REGION 1..107: note = synthetic construct
DIQMTQSPAFLSVSPGERVSFSCRASQNIGTSIHWYQQRTNGSPRLLIKYASESISGIPSRFSGSGSGTDFTLSINSVESEDFADYYCHQSHNWPTTFGAGTKLELK

SEQ ID NO: 203-204 - skipped (2 entries)

SEQ ID NO: 205 - protein, 6 aa, synthetic construct
  REGION 1..6: note = synthetic construct
SGYYWN

SEQ ID NO: 206 - protein, 16 aa, synthetic construct
  REGION 1..16: note = synthetic construct
YITYDGSNNYNPSLKD

SEQ ID NO: 207 - protein, 7 aa, synthetic construct
  REGION 1..7: note = synthetic construct
GGGYVPV

SEQ ID NO: 208 - protein, 11 aa, synthetic construct
  REGION 1..11: note = synthetic construct
RASQNIGTSIH

SEQ ID NO: 209 - protein, 7 aa, synthetic construct
  REGION 1..7: note = synthetic construct
YASESIS

SEQ ID NO: 210 - protein, 9 aa, synthetic construct
  REGION 1..9: note = synthetic construct
HQSHNWPTT

SEQ ID NO: 211 - protein, 8 aa, synthetic construct
  REGION 1..8: note = synthetic construct
GYSITSGY

SEQ ID NO: 212 - protein, 5 aa, synthetic construct
  REGION 1..5: note = synthetic construct
TYDGS

SEQ ID NO: 213 - protein, 7 aa, synthetic construct
  REGION 1..7: note = synthetic construct
GGGYVPV

SEQ ID NO: 214 - protein, 11 aa, synthetic construct
  REGION 1..11: note = synthetic construct
RASQNIGTSIH

SEQ ID NO: 215 - protein, 7 aa, synthetic construct
  REGION 1..7: note = synthetic construct
YASESIS

SEQ ID NO: 216 - protein, 9 aa, synthetic construct
  REGION 1..9: note = synthetic construct
HQSHNWPTT

SEQ ID NO: 217 - protein, 11 aa, synthetic construct
  REGION 1..11: note = synthetic construct
GYSITSGYYWN

SEQ ID NO: 218 - protein, 9 aa, synthetic construct
  REGION 1..9: note = synthetic construct
YITYDGSNN

SEQ ID NO: 219 - protein, 7 aa, synthetic construct
  REGION 1..7: note = synthetic construct
GGGYVPV

SEQ ID NO: 220 - protein, 11 aa, synthetic construct
  REGION 1..11: note = synthetic construct
RASQNIGTSIH

SEQ ID NO: 221 - protein, 7 aa, synthetic construct
  REGION 1..7: note = synthetic construct
YASESIS

SEQ ID NO: 222 - protein, 9 aa, synthetic construct
  REGION 1..9: note = synthetic construct
HQSHNWPTT

SEQ ID NO: 223 - protein, 7 aa, synthetic construct
  REGION 1..7: note = synthetic construct
TSGYYWN

SEQ ID NO: 224 - protein, 12 aa, synthetic construct
  REGION 1..12: note = synthetic construct
WMGYITYDGSNN

SEQ ID NO: 225 - protein, 8 aa, synthetic construct
  REGION 1..8: note = synthetic construct
ARGGGYVP

SEQ ID NO: 226 - protein, 7 aa, synthetic construct
  REGION 1..7: note = synthetic construct
GTSIHWY

SEQ ID NO: 227 - protein, 10 aa, synthetic construct
  REGION 1..10: note = synthetic construct
LLIKYASESI

SEQ ID NO: 228 - protein, 8 aa, synthetic construct
  REGION 1..8: note = synthetic construct
HQSHNWPT

SEQ ID NO: 229 - protein, 9 aa, synthetic construct
  REGION 1..9: note = synthetic construct
GYSITSGYY

SEQ ID NO: 230 - protein, 7 aa, synthetic construct
  REGION 1..7: note = synthetic construct
ITYDGSN

SEQ ID NO: 231 - protein, 9 aa, synthetic construct
  REGION 1..9: note = synthetic construct
ARGGGYVPV

SEQ ID NO: 232 - protein, 6 aa, synthetic construct
  REGION 1..6: note = synthetic construct
QNIGTS

SEQ ID NO: 233 - skipped

SEQ ID NO: 234 - protein, 9 aa, synthetic construct
  REGION 1..9: note = synthetic construct
HQSHNWPTT

SEQ ID NO: 235 - protein, 116 aa, synthetic construct; identical to SEQ ID NO: 167
  REGION 1..116: note = synthetic construct

SEQ ID NO: 236 - protein, 107 aa, synthetic construct
  REGION 1..107: note = synthetic construct
DVQMTQSPAFLSVSPGERVSFSCRASQNIGTSIHWYQQRTNGSPRLLIKYASESISGIPSRFSGSGSGTDFTLSINSVESEDFADYYCHQSHNWPTTFGAGTKLELK

SEQ ID NO: 237-238 - skipped (2 entries)

SEQ ID NO: 239 - protein, 5 aa, synthetic construct
  REGION 1..5: note = synthetic construct
DDNMH

SEQ ID NO: 240 - protein, 17 aa, synthetic construct
  REGION 1..17: note = synthetic construct
YINPNNNHTNYNQKFKG

SEQ ID NO: 241 - protein, 11 aa, synthetic construct
  REGION 1..11: note = synthetic construct
STVVPFYAMDY

SEQ ID NO: 242 - protein, 11 aa, synthetic construct
  REGION 1..11: note = synthetic construct
ITITDIDDDMN

SEQ ID NO: 243 - protein, 7 aa, synthetic construct
  REGION 1..7: note = synthetic construct
EGNTLRP

SEQ ID NO: 244 - protein, 9 aa, synthetic construct
  REGION 1..9: note = synthetic construct
LQSDNLPLT

SEQ ID NO: 245 - protein, 7 aa, synthetic construct
  REGION 1..7: note = synthetic construct
GYTFTDD

SEQ ID NO: 246 - protein, 6 aa, synthetic construct
  REGION 1..6: note = synthetic construct
NPNNNH

SEQ ID NO: 247 - protein, 11 aa, synthetic construct
  REGION 1..11: note = synthetic construct
STVVPFYAMDY

SEQ ID NO: 248 - protein, 11 aa, synthetic construct
  REGION 1..11: note = synthetic construct
ITITDIDDDMN

SEQ ID NO: 249 - protein, 7 aa, synthetic construct
  REGION 1..7: note = synthetic construct
EGNTLRP

SEQ ID NO: 250 - protein, 9 aa, synthetic construct
  REGION 1..9: note = synthetic construct
LQSDNLPLT

SEQ ID NO: 251 - protein, 10 aa, synthetic construct
  REGION 1..10: note = synthetic construct
GYTFTDDNMH

SEQ ID NO: 252 - protein, 10 aa, synthetic construct
  REGION 1..10: note = synthetic construct
YINPNNNHTN

SEQ ID NO: 253 - protein, 11 aa, synthetic construct
  REGION 1..11: note = synthetic construct
STVVPFYAMDY

SEQ ID NO: 254 - protein, 11 aa, synthetic construct
  REGION 1..11: note = synthetic construct
ITITDIDDDMN

SEQ ID NO: 255 - protein, 7 aa, synthetic construct
  REGION 1..7: note = synthetic construct
EGNTLRP

SEQ ID NO: 256 - protein, 9 aa, synthetic construct
  REGION 1..9: note = synthetic construct
LQSDNLPLT

SEQ ID NO: 257 - protein, 6 aa, synthetic construct
  REGION 1..6: note = synthetic construct
TDDNMH

SEQ ID NO: 258 - protein, 13 aa, synthetic construct
  REGION 1..13: note = synthetic construct
WIGYINPNNNHTN

SEQ ID NO: 259 - protein, 12 aa, synthetic construct
  REGION 1..12: note = synthetic construct
ARSTVVPFYAMD

SEQ ID NO: 260 - protein, 7 aa, synthetic construct
  REGION 1..7: note = synthetic construct
DDDMNWY

SEQ ID NO: 261 - protein, 10 aa, synthetic construct
  REGION 1..10: note = synthetic construct
LLFSEGNTLR

SEQ ID NO: 262 - protein, 8 aa, synthetic construct
  REGION 1..8: note = synthetic construct
LQSDNLPL

SEQ ID NO: 263 - protein, 8 aa, synthetic construct
  REGION 1..8: note = synthetic construct
GYTFTDDN

SEQ ID NO: 264 - protein, 8 aa, synthetic construct
  REGION 1..8: note = synthetic construct
INPNNNHT

SEQ ID NO: 265 - protein, 13 aa, synthetic construct
  REGION 1..13: note = synthetic construct
ARSTVVPFYAMDY

SEQ ID NO: 266 - protein, 6 aa, synthetic construct
  REGION 1..6: note = synthetic construct
TDIDDD

SEQ ID NO: 267 - skipped

SEQ ID NO: 268 - protein, 9 aa, synthetic construct
  REGION 1..9: note = synthetic construct
LQSDNLPLT

SEQ ID NO: 269 - protein, 120 aa, synthetic construct
  REGION 1..120: note = synthetic construct
EVQLQESGPELVKPGASVKMSCKASGYTFTDDNMHWVKQSHGKSLEWIGYINPNNNHTNYNQKFKGKATLTVNKSSSTAYMELRSLTSEDSAVYFCARSTVVPFYAMDYWGQGTSVTVSS

SEQ ID NO: 270 - protein, 107 aa, synthetic construct
  REGION 1..107: note = synthetic construct
DIVMTQSPASLSMAIGEKVTIRCITITDIDDDMNWYQQKPGEPPKLLFSEGNTLRPGVPSRFSSSGYGSDFAFTIENMLSEDVADYYCLQSDNLPLTFGAGTKLELK

SEQ ID NO: 271-272 - skipped (2 entries)

SEQ ID NO: 273 - protein, 5 aa, synthetic construct
  REGION 1..5: note = synthetic construct
DDNMH

SEQ ID NO: 274 - protein, 17 aa, synthetic construct
  REGION 1..17: note = synthetic construct
YINPNNNHTNYNQKFKG

SEQ ID NO: 275 - protein, 11 aa, synthetic construct
  REGION 1..11: note = synthetic construct
STVVPFYAMDY

SEQ ID NO: 276 - protein, 11 aa, synthetic construct
  REGION 1..11: note = synthetic construct
ITITDIDDDMN

SEQ ID NO: 277 - protein, 7 aa, synthetic construct
  REGION 1..7: note = synthetic construct
EGNTLRP

SEQ ID NO: 278 - protein, 9 aa, synthetic construct
  REGION 1..9: note = synthetic construct
LQSDNLPLT

SEQ ID NO: 279 - protein, 7 aa, synthetic construct
  REGION 1..7: note = synthetic construct
GYTFTDD

SEQ ID NO: 280 - protein, 6 aa, synthetic construct
  REGION 1..6: note = synthetic construct
NPNNNH

SEQ ID NO: 281 - protein, 11 aa, synthetic construct
  REGION 1..11: note = synthetic construct
STVVPFYAMDY

SEQ ID NO: 282 - protein, 11 aa, synthetic construct
  REGION 1..11: note = synthetic construct
ITITDIDDDMN

SEQ ID NO: 283 - protein, 7 aa, synthetic construct
  REGION 1..7: note = synthetic construct
EGNTLRP

SEQ ID NO: 284 - protein, 9 aa, synthetic construct
  REGION 1..9: note = synthetic construct
LQSDNLPLT

SEQ ID NO: 285 - protein, 10 aa, synthetic construct
  REGION 1..10: note = synthetic construct
GYTFTDDNMH

SEQ ID NO: 286 - protein, 10 aa, synthetic construct
  REGION 1..10: note = synthetic construct
YINPNNNHTN

SEQ ID NO: 287 - protein, 11 aa, synthetic construct
  REGION 1..11: note = synthetic construct
STVVPFYAMDY

SEQ ID NO: 288 - protein, 11 aa, synthetic construct
  REGION 1..11: note = synthetic construct
ITITDIDDDMN

SEQ ID NO: 289 - protein, 7 aa, synthetic construct
  REGION 1..7: note = synthetic construct
EGNTLRP

SEQ ID NO: 290 - protein, 9 aa, synthetic construct
  REGION 1..9: note = synthetic construct
LQSDNLPLT

SEQ ID NO: 291 - protein, 6 aa, synthetic construct
  REGION 1..6: note = synthetic construct
TDDNMH

SEQ ID NO: 292 - protein, 13 aa, synthetic construct
  REGION 1..13: note = synthetic construct
WIGYINPNNNHTN

SEQ ID NO: 293 - protein, 12 aa, synthetic construct
  REGION 1..12: note = synthetic construct
ARSTVVPFYAMD

SEQ ID NO: 294 - protein, 7 aa, synthetic construct
  REGION 1..7: note = synthetic construct
DDDMNWY

SEQ ID NO: 295 - protein, 10 aa, synthetic construct
  REGION 1..10: note = synthetic construct
LLFSEGNTLR

SEQ ID NO: 296 - protein, 8 aa, synthetic construct
  REGION 1..8: note = synthetic construct
LQSDNLPL

SEQ ID NO: 297 - protein, 8 aa, synthetic construct
  REGION 1..8: note = synthetic construct
GYTFTDDN

SEQ ID NO: 298 - protein, 8 aa, synthetic construct
  REGION 1..8: note = synthetic construct
INPNNNHT

SEQ ID NO: 299 - protein, 13 aa, synthetic construct
  REGION 1..13: note = synthetic construct
ARSTVVPFYAMDY

SEQ ID NO: 300 - protein, 6 aa, synthetic construct
  REGION 1..6: note = synthetic construct
TDIDDD

SEQ ID NO: 301 - skipped

SEQ ID NO: 302 - protein, 9 aa, synthetic construct
  REGION 1..9: note = synthetic construct
LQSDNLPLT

SEQ ID NO: 303 - protein, 120 aa, synthetic construct; identical to SEQ ID NO: 269
  REGION 1..120: note = synthetic construct

SEQ ID NO: 304 - protein, 107 aa, synthetic construct
  REGION 1..107: note = synthetic construct
DIQMTQSPASLSMAIGEKVTIRCITITDIDDDMNWYQQKPGEPPKLLFSEGNTLRPGVPSRFSSSGYGSDFAFTIENMLSEDVADYYCLQSDNLPLTFGGGTKLEIK

SEQ ID NO: 305-306 - skipped (2 entries)

SEQ ID NO: 307 - protein, 5 aa, synthetic construct
  REGION 1..5: note = synthetic construct
DDNMH

SEQ ID NO: 308 - protein, 17 aa, synthetic construct
  REGION 1..17: note = synthetic construct
YINPNNNHTNYNQKFKG

SEQ ID NO: 309 - protein, 11 aa, synthetic construct
  REGION 1..11: note = synthetic construct
STVVPFYAMDY

SEQ ID NO: 310 - protein, 11 aa, synthetic construct
  REGION 1..11: note = synthetic construct
ITITDIDDDMN

SEQ ID NO: 311 - protein, 7 aa, synthetic construct
  REGION 1..7: note = synthetic construct
EGNTLRP

SEQ ID NO: 312 - protein, 9 aa, synthetic construct
  REGION 1..9: note = synthetic construct
LQSDNLPLT

SEQ ID NO: 313 - protein, 7 aa, synthetic construct
  REGION 1..7: note = synthetic construct
GYTFTDD

SEQ ID NO: 314 - protein, 6 aa, synthetic construct
  REGION 1..6: note = synthetic construct
NPNNNH

SEQ ID NO: 315 - protein, 11 aa, synthetic construct
  REGION 1..11: note = synthetic construct
STVVPFYAMDY

SEQ ID NO: 316 - protein, 11 aa, synthetic construct
  REGION 1..11: note = synthetic construct
ITITDIDDDMN

SEQ ID NO: 317 - protein, 7 aa, synthetic construct
  REGION 1..7: note = synthetic construct
EGNTLRP

SEQ ID NO: 318 - protein, 9 aa, synthetic construct
  REGION 1..9: note = synthetic construct
LQSDNLPLT

SEQ ID NO: 319 - protein, 10 aa, synthetic construct
  REGION 1..10: note = synthetic construct
GYTFTDDNMH

SEQ ID NO: 320 - protein, 10 aa, synthetic construct
  REGION 1..10: note = synthetic construct
YINPNNNHTN

SEQ ID NO: 321 - protein, 11 aa, synthetic construct
  REGION 1..11: note = synthetic construct
STVVPFYAMDY

SEQ ID NO: 322 - protein, 11 aa, synthetic construct
  REGION 1..11: note = synthetic construct
ITITDIDDDMN

SEQ ID NO: 323 - protein, 7 aa, synthetic construct
  REGION 1..7: note = synthetic construct
EGNTLRP

SEQ ID NO: 324 - protein, 9 aa, synthetic construct
  REGION 1..9: note = synthetic construct
LQSDNLPLT

SEQ ID NO: 325 - protein, 6 aa, synthetic construct
  REGION 1..6: note = synthetic construct
TDDNMH

SEQ ID NO: 326 - protein, 13 aa, synthetic construct
  REGION 1..13: note = synthetic construct
WIGYINPNNNHTN

SEQ ID NO: 327 - protein, 12 aa, synthetic construct
  REGION 1..12: note = synthetic construct
ARSTVVPFYAMD

SEQ ID NO: 328 - protein, 7 aa, synthetic construct
  REGION 1..7: note = synthetic construct
DDDMNWY

SEQ ID NO: 329 - protein, 10 aa, synthetic construct
  REGION 1..10: note = synthetic construct
LLFSEGNTLR

SEQ ID NO: 330 - protein, 8 aa, synthetic construct
  REGION 1..8: note = synthetic construct
LQSDNLPL

SEQ ID NO: 331 - protein, 8 aa, synthetic construct
  REGION 1..8: note = synthetic construct
GYTFTDDN

SEQ ID NO: 332 - protein, 8 aa, synthetic construct
  REGION 1..8: note = synthetic construct
INPNNNHT

SEQ ID NO: 333 - protein, 13 aa, synthetic construct
  REGION 1..13: note = synthetic construct
ARSTVVPFYAMDY

SEQ ID NO: 334 - protein, 6 aa, synthetic construct
  REGION 1..6: note = synthetic construct
TDIDDD

SEQ ID NO: 335 - skipped

SEQ ID NO: 336 - protein, 9 aa, synthetic construct
  REGION 1..9: note = synthetic construct
LQSDNLPLT

SEQ ID NO: 337 - protein, 120 aa, synthetic construct; identical to SEQ ID NO: 269
  REGION 1..120: note = synthetic construct

SEQ ID NO: 338 - protein, 107 aa, synthetic construct
  REGION 1..107: note = synthetic construct
DIKMTQSPASLSMAIGEKVTIRCITITDIDDDMNWYQQKPGEPPKLLFSEGNTLRPGVPSRFSSSGYGSDFAFTIENMLSEDVADYYCLQSDNLPLTFGAGTKLELK

SEQ ID NO: 339-340 - skipped (2 entries)

SEQ ID NO: 341 - protein, 5 aa, synthetic construct
  REGION 1..5: note = synthetic construct
HYWID

SEQ ID NO: 342 - protein, 17 aa, synthetic construct
  REGION 1..17: note = synthetic construct
NIYPGGGYTNYNENFKG

SEQ ID NO: 343 - protein, 13 aa, synthetic construct
  REGION 1..13: note = synthetic construct
KGYYYGSDWYFDV

SEQ ID NO: 344 - protein, 10 aa, synthetic construct
  REGION 1..10: note = synthetic construct
SASSSVSYMH

SEQ ID NO: 345 - protein, 7 aa, synthetic construct
  REGION 1..7: note = synthetic construct
DTSKLAS

SEQ ID NO: 346 - protein, 9 aa, synthetic construct
  REGION 1..9: note = synthetic construct
QQWSSNPYT

SEQ ID NO: 347 - protein, 7 aa, synthetic construct
  REGION 1..7: note = synthetic construct
GYTFTHY

SEQ ID NO: 348 - protein, 6 aa, synthetic construct
  REGION 1..6: note = synthetic construct
YPGGGY

SEQ ID NO: 349 - protein, 13 aa, synthetic construct
  REGION 1..13: note = synthetic construct
KGYYYGSDWYFDV

SEQ ID NO: 350 - protein, 10 aa, synthetic construct
  REGION 1..10: note = synthetic construct
SASSSVSYMH

SEQ ID NO: 351 - protein, 7 aa, synthetic construct
  REGION 1..7: note = synthetic construct
DTSKLAS

SEQ ID NO: 352 - protein, 9 aa, synthetic construct
  REGION 1..9: note = synthetic construct
QQWSSNPYT

SEQ ID NO: 353 - protein, 10 aa, synthetic construct
  REGION 1..10: note = synthetic construct
GYTFTHYWID

SEQ ID NO: 354 - protein, 10 aa, synthetic construct
  REGION 1..10: note = synthetic construct
NIYPGGGYTN

SEQ ID NO: 355 - protein, 13 aa, synthetic construct
  REGION 1..13: note = synthetic construct
KGYYYGSDWYFDV

SEQ ID NO: 356 - protein, 10 aa, synthetic construct
  REGION 1..10: note = synthetic construct
SASSSVSYMH

SEQ ID NO: 357 - protein, 7 aa, synthetic construct
  REGION 1..7: note = synthetic construct
DTSKLAS

SEQ ID NO: 358 - protein, 9 aa, synthetic construct
  REGION 1..9: note = synthetic construct
QQWSSNPYT

SEQ ID NO: 359 - protein, 6 aa, synthetic construct
  REGION 1..6: note = synthetic construct
THYWID

SEQ ID NO: 360 - protein, 13 aa, synthetic construct
  REGION 1..13: note = synthetic construct
WIGNIYPGGGYTN

SEQ ID NO: 361 - protein, 14 aa, synthetic construct
  REGION 1..14: note = synthetic construct
TRKGYYYGSDWYFD

SEQ ID NO: 362 - protein, 6 aa, synthetic construct
  REGION 1..6: note = synthetic construct
SYMHWY

SEQ ID NO: 363 - protein, 10 aa, synthetic construct
  REGION 1..10: note = synthetic construct
RWIYDTSKLA

SEQ ID NO: 364 - protein, 8 aa, synthetic construct
  REGION 1..8: note = synthetic construct
QQWSSNPY

SEQ ID NO: 365 - protein, 8 aa, synthetic construct
  REGION 1..8: note = synthetic construct
GYTFTHYW

SEQ ID NO: 366 - protein, 8 aa, synthetic construct
  REGION 1..8: note = synthetic construct
IYPGGGYT

SEQ ID NO: 367 - protein, 15 aa, synthetic construct
  REGION 1..15: note = synthetic construct
TRKGYYYGSDWYFDV

SEQ ID NO: 368 - protein, 5 aa, synthetic construct
  REGION 1..5: note = synthetic construct
SSVSY

SEQ ID NO: 369 - skipped

SEQ ID NO: 370 - protein, 9 aa, synthetic construct
  REGION 1..9: note = synthetic construct
QQWSSNPYT

SEQ ID NO: 371 - protein, 122 aa, synthetic construct; identical to SEQ ID NO: 65
  REGION 1..122: note = synthetic construct

SEQ ID NO: 372 - protein, 106 aa, synthetic construct
  REGION 1..106: note = synthetic construct
QIVLSQSPAIMSASPGEKVTMTCSASSSVSYMHWYQQKSGTSPKRWIYDTSKLASGVPARFSGSGSGTSYSLTISSMEAEDAATYYCQQWSSNPYTFGGGTKLEIK

SEQ ID NO: 373-374 - skipped (2 entries)

SEQ ID NO: 375 - protein, 6 aa, synthetic construct
  REGION 1..6: note = synthetic construct
SGYYWK

SEQ ID NO: 376 - protein, 16 aa, synthetic construct
  REGION 1..16: note = synthetic construct
YISYDGSNNYNPSLKN

SEQ ID NO: 377 - protein, 7 aa, synthetic construct
  REGION 1..7: note = synthetic construct
GGGYVPV

SEQ ID NO: 378 - protein, 16 aa, synthetic construct
  REGION 1..16: note = synthetic construct
RSSQSIVRSNGNTYLE

SEQ ID NO: 379 - protein, 7 aa, synthetic construct
  REGION 1..7: note = synthetic construct
KVSNRFS

SEQ ID NO: 380 - protein, 9 aa, synthetic construct
  REGION 1..9: note = synthetic construct
FQSSHVPRT

SEQ ID NO: 381 - protein, 8 aa, synthetic construct
  REGION 1..8: note = synthetic construct
GYFISSGY

SEQ ID NO: 382 - protein, 5 aa, synthetic construct
  REGION 1..5: note = synthetic construct
SYDGS

SEQ ID NO: 383 - protein, 7 aa, synthetic construct
  REGION 1..7: note = synthetic construct
GGGYVPV

SEQ ID NO: 384 - protein, 16 aa, synthetic construct
  REGION 1..16: note = synthetic construct
RSSQSIVRSNGNTYLE

SEQ ID NO: 385 - protein, 7 aa, synthetic construct
  REGION 1..7: note = synthetic construct
KVSNRFS

SEQ ID NO: 386 - protein, 9 aa, synthetic construct
  REGION 1..9: note = synthetic construct
FQSSHVPRT

SEQ ID NO: 387 - protein, 11 aa, synthetic construct
  REGION 1..11: note = synthetic construct
GYFISSGYYWK

SEQ ID NO: 388 - protein, 9 aa, synthetic construct
  REGION 1..9: note = synthetic construct
YISYDGSNN

SEQ ID NO: 389 - protein, 7 aa, synthetic construct
  REGION 1..7: note = synthetic construct
GGGYVPV

SEQ ID NO: 390 - protein, 16 aa, synthetic construct
  REGION 1..16: note = synthetic construct
RSSQSIVRSNGNTYLE

SEQ ID NO: 391 - protein, 7 aa, synthetic construct
  REGION 1..7: note = synthetic construct
KVSNRFS

SEQ ID NO: 392 - protein, 9 aa, synthetic construct
  REGION 1..9: note = synthetic construct
FQSSHVPRT

SEQ ID NO: 393 - protein, 7 aa, synthetic construct
  REGION 1..7: note = synthetic construct
SSGYYWK

SEQ ID NO: 394 - protein, 12 aa, synthetic construct
  REGION 1..12: note = synthetic construct
WMGYISYDGSNN

SEQ ID NO: 395 - protein, 8 aa, synthetic construct
  REGION 1..8: note = synthetic construct
ARGGGYVP

SEQ ID NO: 396 - protein, 12 aa, synthetic construct
  REGION 1..12: note = synthetic construct
VRSNGNTYLEWY

SEQ ID NO: 397 - protein, 10 aa, synthetic construct
  REGION 1..10: note = synthetic construct
LLIYKVSNRF

SEQ ID NO: 398 - protein, 8 aa, synthetic construct
  REGION 1..8: note = synthetic construct
FQSSHVPR

SEQ ID NO: 399 - protein, 9 aa, synthetic construct
  REGION 1..9: note = synthetic construct
GYFISSGYY

SEQ ID NO: 400 - protein, 7 aa, synthetic construct
  REGION 1..7: note = synthetic construct
ISYDGSN

SEQ ID NO: 401 - protein, 9 aa, synthetic construct
  REGION 1..9: note = synthetic construct
ARGGGYVPV

SEQ ID NO: 402 - protein, 11 aa, synthetic construct
  REGION 1..11: note = synthetic construct
QSIVRSNGNTY

SEQ ID NO: 403 - skipped

SEQ ID NO: 404 - protein, 9 aa, synthetic construct
  REGION 1..9: note = synthetic construct
FQSSHVPRT

SEQ ID NO: 405 - protein, 116 aa, synthetic construct
  REGION 1..116: note = synthetic construct
EVQLQESGPGLVKPSQSLSLTCSVTGYFISSGYYWKWIRQFPGNKLEWMGYISYDGSNNYNPSLKNRISITRDTSKNQFFLKLNSVTAEDTATYYCARGGGYVPVWGTGTTVTVSS

SEQ ID NO: 406 - protein, 112 aa, synthetic construct
  REGION 1..112: note = synthetic construct
DIQMTQSPLSLPVSLGDQASISCRSSQSIVRSNGNTYLEWYLQKPGQSPKLLIYKVSNRFSGVPDRFSGSGSGTDFTLKISRVEAEDLGVYYCFQSSHVPRTFGGGTKLEIK

SEQ ID NO: 407-408 - skipped (2 entries)

SEQ ID NO: 409 - protein, 6 aa, synthetic construct
  REGION 1..6: note = synthetic construct
SGYYWK

SEQ ID NO: 410 - protein, 16 aa, synthetic construct
  REGION 1..16: note = synthetic construct
YISYDGSNNYNPSLKN

SEQ ID NO: 411 - protein, 7 aa, synthetic construct
  REGION 1..7: note = synthetic construct
GGGYVPV

SEQ ID NO: 412 - protein, 16 aa, synthetic construct
  REGION 1..16: note = synthetic construct
RSSQSIVRSNGNTYLE

SEQ ID NO: 413 - protein, 7 aa, synthetic construct
  REGION 1..7: note = synthetic construct
KVSNRFS

SEQ ID NO: 414 - protein, 9 aa, synthetic construct
  REGION 1..9: note = synthetic construct
FQSSHVPRT

SEQ ID NO: 415 - protein, 8 aa, synthetic construct
  REGION 1..8: note = synthetic construct
GYFISSGY

SEQ ID NO: 416 - protein, 5 aa, synthetic construct
  REGION 1..5: note = synthetic construct
SYDGS

SEQ ID NO: 417 - protein, 7 aa, synthetic construct
  REGION 1..7: note = synthetic construct
GGGYVPV

SEQ ID NO: 418 - protein, 16 aa, synthetic construct
  REGION 1..16: note = synthetic construct
RSSQSIVRSNGNTYLE

SEQ ID NO: 419 - protein, 7 aa, synthetic construct
  REGION 1..7: note = synthetic construct
KVSNRFS

SEQ ID NO: 420 - protein, 9 aa, synthetic construct
  REGION 1..9: note = synthetic construct
FQSSHVPRT

SEQ ID NO: 421 - protein, 11 aa, synthetic construct
  REGION 1..11: note = synthetic construct
GYFISSGYYWK

SEQ ID NO: 422 - protein, 9 aa, synthetic construct
  REGION 1..9: note = synthetic construct
YISYDGSNN

SEQ ID NO: 423 - protein, 7 aa, synthetic construct
  REGION 1..7: note = synthetic construct
GGGYVPV

SEQ ID NO: 424 - protein, 16 aa, synthetic construct
  REGION 1..16: note = synthetic construct
RSSQSIVRSNGNTYLE

SEQ ID NO: 425 - protein, 7 aa, synthetic construct
  REGION 1..7: note = synthetic construct
KVSNRFS

SEQ ID NO: 426 - protein, 9 aa, synthetic construct
  REGION 1..9: note = synthetic construct
FQSSHVPRT

SEQ ID NO: 427 - protein, 7 aa, synthetic construct
  REGION 1..7: note = synthetic construct
SSGYYWK

SEQ ID NO: 428 - protein, 12 aa, synthetic construct
  REGION 1..12: note = synthetic construct
WMGYISYDGSNN

SEQ ID NO: 429 - protein, 8 aa, synthetic construct
  REGION 1..8: note = synthetic construct
ARGGGYVP

SEQ ID NO: 430 - protein, 12 aa, synthetic construct
  REGION 1..12: note = synthetic construct
VRSNGNTYLEWY

SEQ ID NO: 431 - protein, 10 aa, synthetic construct
  REGION 1..10: note = synthetic construct
LLIYKVSNRF

SEQ ID NO: 432 - protein, 8 aa, synthetic construct
  REGION 1..8: note = synthetic construct
FQSSHVPR

SEQ ID NO: 433 - protein, 9 aa, synthetic construct
  REGION 1..9: note = synthetic construct
GYFISSGYY

SEQ ID NO: 434 - protein, 7 aa, synthetic construct
  REGION 1..7: note = synthetic construct
ISYDGSN

SEQ ID NO: 435 - protein, 9 aa, synthetic construct
  REGION 1..9: note = synthetic construct
ARGGGYVPV

SEQ ID NO: 436 - protein, 11 aa, synthetic construct
  REGION 1..11: note = synthetic construct
QSIVRSNGNTY

SEQ ID NO: 437 - skipped

SEQ ID NO: 438 - protein, 9 aa, synthetic construct
  REGION 1..9: note = synthetic construct
FQSSHVPRT

SEQ ID NO: 439 - protein, 116 aa, synthetic construct; identical to SEQ ID NO: 405
  REGION 1..116: note = synthetic construct

SEQ ID NO: 440 - protein, 112 aa, synthetic construct
  REGION 1..112: note = synthetic construct
DIKMTQSPLSLPVSLGDQASISCRSSQSIVRSNGNTYLEWYLQKPGQSPKLLIYKVSNRFSGVPDRFSGSGSGTDFTLKISRVEAEDLGVYYCFQSSHVPRTFGGGTKLEIK